European Patent Application EP 4 286 518 A1, published December 6, 2023. Title: TUMOR-TARGETING TRANS-SPLICING RIBOZYME EXPRESSING IMMUNE CHECKPOINT INHIBITOR AND USE THEREOF. Applicant: RZNOMICS INC. The sequence listing filed with the application follows.

SEQUENCE LISTING (10 sequences)

SEQ ID NO: 1 - DNA, 744 bp, Artificial Sequence
  gene encoding scFv PD1(I)
caggtacaacttgttcagtccggagctgaagtgaaaaagccgggcgcgtctgttaaggtaagctgcaaggcttcaggctatactttcacggcgcagtacatgcattgggtcagacaagctccaggccaaggtcttgaatggatggggatcatcaacccgagtgggggtgaaacaggctatgctcaaaagttccagggtcgagtcaccatgactcgggatacctccacgtctaccgtttacatggagctgagcagtttgaggagcgaagatactgccgtatactattgtgccaaggaaggtgttgcggacggttatgggctcgttgatgtatgggggcaaggcacgatggttaccgtctcatctggtggaggaggttctgggggtggaggctcaggaggaggggggtcaggtggcggaggatccgaaatcgtgttgacccagagtcctgcaacactgagtctgtccccaggggagagagccaccttgtcctgtagagcgagccagtctgtaagctcttatctggcttggtatcagcaaaaacctgggcaggcgccgcgcctcctcatctatgacgcgagcaagagggcaacagggataccagcgagattctctgggtcaggatcagggacagacttcacactcacgatcagctctttggaaccagaagattttgcagtctactattgtgatcaacgaaacaactggcctctcacgttcggaggagggactaaagtagaaattaaa

SEQ ID NO: 2 - DNA, 720 bp, Artificial Sequence
  gene encoding scFv PD1(N)
caggtccaacttgtcgagagcggcggtggagtggtacagcctgggcgatccttgcggcttgattgcaaggcgagcggaataaccttcagcaacagtgggatgcactgggtaagacaagcgccaggcaaggggctcgagtgggtcgctgtcatctggtatgacggaagtaaacgatattacgccgatagtgtaaagggaaggtttacgatcagtagggataactctaaaaatacgctctttcttcaaatgaacagtcttcgagcagaagatacagcggtgtattattgtgctactaatgacgattattggggccagggtactctcgttacggtaagctctggtggaggaggaagtggtggcggaggtagtggaggtggcggctccgggggtggaggatccgagatagtactcacacaaagtcctgctacgctttcactctcccctggagagagagctactctctcatgccgagcctcccagagtgtgagttcatatttggcgtggtaccagcagaagcccggccaagccccccgattgctcatatatgacgccagtaatcgcgcgactggtatacctgcccggtttagcggaagtggatccgggacggactttaccctgacaatttcttcactggagcctgaagacttcgccgtatattattgtcaacaatcctccaattggccaagaacttttggccaaggaacgaaagttgagataaaa

SEQ ID NO: 3 - DNA, 735 bp, Artificial Sequence
  gene encoding scFv PDL1(A)
gaagttcaactggtggagtctggagggggtttggtgcagccaggcgggagtttgaggctcagctgcgccgcctctggattcaccttctccgatagctggatccattgggtcaggcaagcgcctggtaaagggttggagtgggtcgcatggatatctccttatggagggtctacatattatgccgactctgtcaagggaagattcacgatatccgcagacacaagtaagaatacagcataccttcaaatgaactccctgcgcgctgaagacacggcggtttattattgcgctaggcggcactggccagggggttttgactattggggtcaaggtaccttggtcacggtttcatccggcggcggtggtagcggtggtggaggtagcgggggtggtggaagtgggggtggaggctcagacatccaaatgacacaaagcccatcctccctgagcgctagtgtgggggaccgggtcacgataacctgccgggctagccaagatgtgagcacagcagtcgcctggtatcagcagaagcccgggaaggccccaaaactcctcatatactctgcttcttttctctattccggtgtgccctctcgattctcaggcagtgggtcaggaaccgacttcacgctgaccatctcaagtttgcagccggaagacttcgcaacgtattattgccagcaatacctctaccatcctgccactttcggtcaggggacgaaagtagagattaaa

SEQ ID NO: 4 - DNA, 393 bp, Artificial Sequence
  sequence encoding hTERT targeting ribozyme
ggcaggaaaagttatcaggcatgcacctggtagctagtctttaaaccaatagattgcatcggtttaaaaggcaagaccgtcaaattgcgggaaaggggtcaacagccgttcagtaccaagtctcaggggaaactttgagatggccttgcaaagggtatggtaataagctgacggacatggtcctaaccacgcagccaagtcctaagtcaacagatcttctgttgatatggatgcagttcacagactaaatgtcggtcggggaagatgtattcttctcataagatatagtcggacctctccttaatgggagctagcggatgaagtgatgcaacactggagccgctgggaactaatttgtatgcgaaagtatattgattagttttggagtactcg

SEQ ID NO: 5 - DNA, 1128 bp, Artificial Sequence
  sequence encoding HSVkt
atggcttcgtacccctgccatcaacacgcgtctgcgttcgaccaggctgcgcgttctcgcggccatagcaaccgacgtacggcgttgcgccctcgccggcagcaagaagccacggaagtccgcctggagcagaaaatgcccacgctactgcgggtttatatagacggtcctcacgggatggggaaaaccaccaccacgcaactgctggtggccctgggttcgcgcgacgatatcgtctacgtacccgagccgatgacttactggcaggtgctgggggcttccgagacaatcgcgaacatctacaccacacaacaccgcctcgaccagggtgagatatcggccggggacgcggcggtggtaatgacaagcgcccagataacaatgggcatgccttatgccgtgaccgacgccgttctggctcctcatatcgggggggaggctgggagctcacatgccccgcccccggccctcaccctcatcttcgaccgccatcccatcgccgccctcctgtgctacccggccgcgcgataccttatgggcagcatgaccccccaggccgtgctggcgttcgtggccctcatcccgccgaccttgcccggcacaaacatcgtgttgggggcccttccggaggacagacacatcgaccgcctggccaaacgccagcgccccggcgagcggcttgacctggctatgctggccgcgattcgccgcgtttacgggctgcttgccaatacggtgcggtatctgcagggcggcgggtcgtggcgggaggattggggacagctttcggggacggccgtgccgccccagggtgccgagccccagagcaacgcgggcccacgaccccatatcggggacacgttatttaccctgtttcgggcccccgagttgctggcccccaacggcgacctgtacaacgtgtttgcctgggccttggacgtcttggccaaacgcctccgtcccatgcacgtctttatcctggattacgaccaatcgcccgccggctgccgggacgccctgctgcaacttacctccgggatggtccagacccacgtcaccacccccggctccataccgacgatctgcgacctggcgcgcacgtttgcccgggagatgggggaggctaac

SEQ ID NO: 6 - DNA, 22 bp, Artificial Sequence
  sequence encoding miR-122T
caaacaccattgtcacactcca

SEQ ID NO: 7 - DNA, 57 bp, Artificial Sequence
  sequence encoding p2a
gccacaaacttctctctgctaaagcaagcaggtgatgttgaagaaaaccccgggcct

SEQ ID NO: 8 - DNA, 19 bp, Artificial Sequence
  RT primer(HSV-tk) of primer premix
agttagcctcccccatctc

SEQ ID NO: 9 - DNA, 25 bp, Artificial Sequence
  hTERT primer of primer premix
ggaattcgcagcgctgcgtcctgct

SEQ ID NO: 10 - DNA, 30 bp, Artificial Sequence
  HSVkt primer of primer premix
gtgaggaccgtctatataaacccgcagtag